European Patent Specification EP 3 365 371 B1, published October 8, 2025. Title: GITR AGONISTS. Applicant: Ablynx NV. The sequence listing filed with the application follows.

SEQUENCE LISTING (292 sequences)

SEQ ID NO: 1 - protein, 121 aa, Artificial Sequence
  Nanobody Sequence
EVQLVESGGGLVQPGGSLRLSCAASETIFSIDSMAWYRQAPGKQRELVAAITGGGSPNYADSVKGRFTISSDVAKRTVYLQMNSLKPEDTAVYYCNAEGQAGWGTALMDYWGKGTLVTVSS

SEQ ID NO: 2 - protein, 121 aa, Artificial Sequence
  Nanobody Sequence
EVQLVESGGGLVQPGGSLRLSCTASESIFSIDAMGWHRQAPGKQRELVAHITGGGRSNYADSVKGRFTISGDSAKRTVYLQMNSLKPEDTAVYYCNAEGQAGWGTALMDYWGKGTLVTVSS

SEQ ID NO: 3 - protein, 121 aa, Artificial Sequence
  Nanobody Sequence
EVQLVESGGGLVQPGGSLRLSCAASESIFSIDAMGWYHQAPGKQRELVATITGGGSTNYADSVKGRFTISGDSAKRTVYLQMDSLKPEDTAVYYCNAEGQAGWGTALMDYWGKGTLVTVSS

SEQ ID NO: 4 - protein, 121 aa, Artificial Sequence
  Nanobody Sequence
EVQLVESGGGLVQSGGSLRLSCAASESIFSIDAMGWYRQAPGKQRELVATITGGGRRNYADSVMGRFSISGDNAKRTVYLQMNSLKPEDTAVYYCNAEGQAGWGTALMDYWGKGTQVTVSS

SEQ ID NO: 5 - protein, 121 aa, Artificial Sequence
  Nanobody Sequence
EVQLVESGGGLVQPGGSLRLSCAASESIFSIDAMGWHRQAPGKQRELVAHITGGGRSNYADSVKGRFTISGDSAKRTVYLQMNSLKPEDTAVYYCNAEGQAGWGTALMDYWGKGTQVTVSS

SEQ ID NO: 6 - protein, 121 aa, Artificial Sequence
  Nanobody Sequence
EVQLVESGGGLVQPGGSLRLSCTASESIFSIDAMGWHRQAPGKQRELVAHITGGGRSNYADSVKGRFTISGDSAKRTVYLQMNSLRPEDTAVYYCNAEGQAGWGTALMDYWGKGTLVTVSS

SEQ ID NO: 7 - protein, 121 aa, Artificial Sequence
  Nanobody Sequence
EVQLVESGGGLVRPGGSLRLSCAASESIFSIDAMGWYRQAPGKQRELVATMTGGGSTNYADSVKGRFTISSDVAKRTVYLQMNSLKPEDTAVYYCNAEGQAGWGTALMDYWGKGTQVTVSS

SEQ ID NO: 8 - protein, 121 aa, Artificial Sequence
  Nanobody Sequence
EVQLVESGGGLVQPGGSLRLSCTASESIFSIDAMGWHRQAPGKQRELVAHITGGGGSNYADSVKGRFTISGDSAKRTVYLQMNSLKPEDTAVYYCNAEGQAGWGTALMDYWGKGTQVTVSS

SEQ ID NO: 9 - protein, 121 aa, Artificial Sequence
  Nanobody Sequence
EVQLVESGGGLVQPGGSLRLSCAASETIFSIDSMAWYRQAPGRQRELVAAITGGGSPNYADSVKGRFTISSDVAKRTVYLQMNSLKPEDTAVYYCNAEGQAGWGTALMDYWGKGTLVTVSS

SEQ ID NO: 10 - protein, 121 aa, Artificial Sequence
  Nanobody Sequence
EVQLVESGGGLVQPGGSLRLSCAASETIFSIDSMAWYRQAPGKQRELVAAITGGGSPNYADSVKGRFTISSDVAKRTAYLQMNSLKPEDTAVYYCNAEGQAGWGTALMDYWGKGTLVTVSS

SEQ ID NO: 11 - protein, 121 aa, Artificial Sequence
  Nanobody Sequence
EVQLVESGGGLVRPGGSLRLSCAASESIFSIDAMGWYRQAPGKQRELVATMTGGGSTNYADSVRGRFTISSDVAKRTVYLQMNSLKPEDTAVYYCNAEGQAGWGTALMDYWGKGTQVTVSS

SEQ ID NO: 12 - protein, 121 aa, Artificial Sequence
  Nanobody Sequence
EVQLVESGGGLVQPGGSLRLSCTASESIFSIDAMGWHRQAPGKQRELVAHITGGGRSNYADSVKGRFAISGDSAKRTVYLQMNSLKPEDTAVYYCNAEGQAGWGTALMDYWGKGTQVTVSS

SEQ ID NO: 13 - protein, 121 aa, Artificial Sequence
  Nanobody Sequence
EVQLVESGGGLVQPGGSLRLSCAASESIFSIDAMGWYRQAPGKQRELVATITGGGSTNYADSVKGRFTISGDSAKRTVYLQMDSLKPEDTAVYYCNAEGQAGWGTALMDYWGKGTLVTVSS

SEQ ID NO: 14 - protein, 121 aa, Artificial Sequence
  Nanobody Sequence
EVQLVESGGGLVRPGGSLRLPCAASESIFSIDAMGWYRQAPGKQRELVATMTGGGSTNYADSVKGRFTISSDVAKRTVYLQMNSLKPEDTAVYYCNAEGQAGWGTALMDYWGKGTLVTVSS

SEQ ID NO: 15 - protein, 121 aa, Artificial Sequence
  Nanobody Sequence
EVQLVESGGGLVQSGGSLRLSCAASESIFSINAMGWYRQAPGKQRELVATITGGGRRNYADSVMGRFSISGDNAKRTVYLQMNSLKPEDTAVYYCNAEGQAGWGTALMDYWGKGTQVTVSS

SEQ ID NO: 16 - protein, 121 aa, Artificial Sequence
  Nanobody Sequence
EVQLVESGGGLVQPGGSLRLSCAASESIFSIDAMGWYRQAPGKQRELVATITGGSSTNYADSVKGRFTISGDNAKRTVYLQMNSLKPEDTAVYYCNAEGQAGWGTALMDYWGKGTQVTVSS

SEQ ID NO: 17 - protein, 121 aa, Artificial Sequence
  Nanobody Sequence
EVQLVESGGGLVQPGGSLRLSCAASESIFSIDAMGWYRQAPGKQRELVATITGGGSTNYADSVKGRFTISGDNAKRTVYLQMNSLKPEDTAAYYCNAEGQAGWGTALMDYWGKGTLVTVSS

SEQ ID NO: 18 - protein, 121 aa, Artificial Sequence
  Nanobody Sequence
EVQLVESGGGLVQPGGSLRLSCTASESIFSIDAMGWHRQAPGKQRELVAHITGGGRSNYADSVKGRFTISGDSAKRTVYLQMNSLKPGDTAVYYCNAEGQAGWGTALMDYWGKGTQVTVSS

SEQ ID NO: 19 - protein, 121 aa, Artificial Sequence
  Nanobody Sequence
EVQLVESGGGLVQPGGSLRLSCAASESIFSIDAMGWYRQAPGKQRELVATITGGGSTNYADSVKGRFTISGDNAKRTVYLQMNSLKPEDTAVYYCNAEGQAGWGTALMDYWGKGTQVTVSS

SEQ ID NO: 20 - protein, 121 aa, Artificial Sequence
  Nanobody Sequence
EVQLVESGGGLVQPGGSLRLSCTASESIFSIDAMGWHRQAPGKQRELVAHITGGGRPNYADSVKGRFTISGDSAKRTVYLQMNSLKPEDTAVYYCNAEGQAGWGTALMDYWGKGTLVTVSS

SEQ ID NO: 21 - protein, 121 aa, Artificial Sequence
  Nanobody Sequence
EVQLVESGGGLVQPGGSLRLSCAGSESIFSIDAMGWYRQAPGKQRELVAGISGGGRTNYADSVKGRFTISGDNAKNTVYLQMNSLKPEDTAVYYCNAEGQAGWGTPLMNYWGKGTLVTVSS

SEQ ID NO: 22 - protein, 119 aa, Artificial Sequence
  Nanobody Sequence
EVQLVESGGGLVQPGGSLRLSCAASGSIFSIDSMGWYRQAPGKQRELVAAITSSTNYADSVKGRFTISRDNAKNTVYLQMNSLKPEDTAVYYCNLEGQAGWGTALINYWGKGTLVTVSS

SEQ ID NO: 23 - protein, 119 aa, Artificial Sequence
  Nanobody Sequence
EVQLVESGGGLVQPGGSLRLTCAASGSIFSIDAMGWYRQAPGKQRELVASITSTTNYAESVKGRFTISRANAKNTVYLQMNSLKPEDTAVYYCNVKGQTGWGTALMDYWGKGTQVTVSS

SEQ ID NO: 24 - protein, 119 aa, Artificial Sequence
  Nanobody Sequence
EVQLVESGGGLVQPGGSLRLTCAASGSIFSIDAMGWYRQAPGKQRELVASITSTTNYAESVKGRFTISRANAKNTVYLQMNSLKPEDTAVYYCSVKGQTGWGTALMDYWGKGTLVTVSS

SEQ ID NO: 25 - protein, 119 aa, Artificial Sequence
  Nanobody Sequence
EVQLVESGGGLVQPGGSLRLSCAASGSIFSINAMGWYRQAPGKQRELVAAITSGTNYADSAKGRFTISRDHAKNTVYLQMNSLKPEDTAVYYCNLEGQTGWGTALMDYWGKGTLVTVSS

SEQ ID NO: 26 - protein, 119 aa, Artificial Sequence
  Nanobody Sequence
EVQLVESGGGLVQPGGSLRLSCAASGSIFSINAMGWYRQAPGKQRELVAAITSGTNYADSVKGRFTISRDHAKNTVYLQMNSLKPEDTAVYYCNLEGQTGWGTALMDYWGKGTQVTVSS

SEQ ID NO: 27 - protein, 119 aa, Artificial Sequence
  Nanobody Sequence
EVQLVESGGGLVQPGGSLRLFCAASGSIFSINAMGWYRQAPGKQRELVAAITSGTNYADSVRGRFTISRDHAKNTVYLQMNSLKPEDTAVYYCNLEGQTGWGTALMDYWGKGTQVTVSS

SEQ ID NO: 28 - protein, 119 aa, Artificial Sequence
  Nanobody Sequence
EVQLVESGGGLVQPGGSLRLSCAASGSIFSINAMGWYRQAPGKQRELVAAITSGTNYADSVKGRFTISRDHAKNTVYLQMNSLKPEDTAVYYCNLEGQTGWGTALMDYWGKGTLVTVSS

SEQ ID NO: 29 - protein, 119 aa, Artificial Sequence
  Nanobody Sequence
EVQLVESGGGLVQPGGSLRLSCAASGSIFSIDSMGWYRQAPGKQRELVAAITSRTIYADSVKGRFTISRDNAKNTVYLQMNSLKPEDTAVYYCNLEGQAGWGTALMDYWGKGTLVTVSS

SEQ ID NO: 30 - protein, 119 aa, Artificial Sequence
  Nanobody Sequence
EVQLVESGGGLVQPGGSLRLSCAASGSIFSIDAMGWYRQAPGKQRELVATITSGKNYADSVKGRFTISRDNAKNAVYLQMNSLKPEDTAVYYCNLEGQAGWGTALMDYWGKGTQVTVSS

SEQ ID NO: 31 - protein, 119 aa, Artificial Sequence
  Nanobody Sequence
EVQLVESGGGLVQPGGSLRLSCAASGSIFSIDSMGWYRQAPGKQRELVAAITSSTNYADSVKGRFTISRDNAKNTVYLQTNSLKPEDTAVYYCNLEGQAGWGTALMDYWGKGTQVTVSS

SEQ ID NO: 32 - protein, 119 aa, Artificial Sequence
  Nanobody Sequence
EVQLVESGGGLVQPGGSLRLSCAASGSIFSINAMGWYRQAPGKQRELVAAITSSTNYADSVKGRFTISRANAKNTVYLQMNSLKPEDTAVYYCHLEGQAGWGTALLDYWGKGTLVTVSS

SEQ ID NO: 33 - protein, 121 aa, Artificial Sequence
  Nanobody Sequence
EVQLVESGGDLVQPGGSLRLSCAASGSVFSINDMGWFRQAPGKQRELVADIISRGVTNYADSVKGRFTISGDPAKNTVYLQMNSLKPEDTAVYYCNAHISTGWGRPHNNYWGQGTQVTVSS

SEQ ID NO: 34 - protein, 121 aa, Artificial Sequence
  Nanobody Sequence
EVQLVESGGDLVQPGGSLRLSCAASGSIFSIDSMGWFRQAPGKQRELVADIISADVTNYADSVKGRFTISGDHAKNTVYLQMNSLKPEDTAVYYCNAHISTGWGRPHNNYWGQGTQVTVSS

SEQ ID NO: 35 - protein, 121 aa, Artificial Sequence
  Nanobody Sequence
EVQLVESGGDLVQPGGSLRLSCAASGSIFSIDSMGWFRQAPGKQRELVADIISADVTNYADSVKGRFTISGDHAQNTVYLQMNSLKPEDTAVYYCNAHISTGWGRPHNNYWGQGTQVTVSS

SEQ ID NO: 36 - protein, 121 aa, Artificial Sequence
  Nanobody Sequence
EVQLVESGGDLVQPGGSLRLSCAASGSIFSIDSMGWFRQAPGKQRELVADIISAGVTNYADSVKGRFTISGDHAKNTVYLQMNSLKPEDTAVYYCNAHISTGWGRPHNNYWGQGTQVTVSS

SEQ ID NO: 37 - protein, 121 aa, Artificial Sequence
  Nanobody Sequence
EVQLVESGGDLVQPGGSLRLSCAASGSIFSIDDMGWFRQAPGKQRELVADIISAGVTNYADSVKGRFTISGDHAKNTVYLQMNSLKPEDTAVYYCNAHISTGWGRPHNNYWGQGTLVTVSS

SEQ ID NO: 38 - protein, 121 aa, Artificial Sequence
  Nanobody Sequence
EVQLVESGGDLVQPGGSLRLSCAASGSIFSINDVGWFRQAPGKQRELVADIISRGVTNYADSVKGRFTISGDPAKNTVYLQMNSLKPEDTAAYYCNAHISTGWGRPHNNYWGQGTQVTVSS

SEQ ID NO: 39 - protein, 121 aa, Artificial Sequence
  Nanobody Sequence
EVQLVESGGDLVQPGGPLRLSCAASGNIFSINDMGWFRQAPGKQRELVADIISRGVTNYADSVKGRFTISGDPAKNTVYLQMNSLKPEDTAVYYCNAHISTGWGRPHNNYWGQGTQVTVSS

SEQ ID NO: 40 - protein, 121 aa, Artificial Sequence
  Nanobody Sequence
EVQLVESGGDLVQPGGPLRLSCAASGSIFSINDMGWFRQAPGKQRELVADIISRGVTNYADSVKGRFTISGDPAKNTVYLQMNSLKPEDTAVYYCNAHISTGWGRPHNNYWGQGTQVTVSS

SEQ ID NO: 41 - protein, 121 aa, Artificial Sequence
  Nanobody Sequence
EVQLVESGGDLVQPGGSLRLSCAASGSIFSINDMGWFRQAPGKQRELVADIISRGVTNYADSVKGRFTISGDPAKNTVYLQMNSLKPEDTAVYYCNAHISTGWGRPHNNYWGQGTQVTVSS

SEQ ID NO: 42 - protein, 121 aa, Artificial Sequence
  Nanobody Sequence
EVQLVESGGDLVQPGGSLRLSCAASGSIFSINDTGWFRQAPGKQRELVADIISRGVTNYADSVKGRFTISGDPAKNTVYLQMNSLKPEDTAVYYCNAHISTGWGRPHNNYWGQGTQVTVSS

SEQ ID NO: 43 - protein, 121 aa, Artificial Sequence
  Nanobody Sequence
EVQLVESGGDLVQPGGSLRLSCAASGSIFSINDMGWFRQAPGKQRELVADIISAGVTNYADSVKGRFTISGDPAKNTVYLQMNSLKPEDTAVYYCNAHISTGWGRPHNNYWGQGTQVTVSS

SEQ ID NO: 44 - protein, 121 aa, Artificial Sequence
  Nanobody Sequence
EVQLVESGGDLVQPGGSLRLSCAASGSIFSINDMGWFRQAPGKQRELVAGIISRGVTNYADSVKGRFTISGDPAKNTVYLQMNSLKPEDTAVYYCNAHISTGWGRPHNNYWGQGTQVTVSS

SEQ ID NO: 45 - protein, 121 aa, Artificial Sequence
  Nanobody Sequence
EVQLVESGGDLVQPGGSLRLSCAASGSIFSINDMGWFRQAPGKQRELVADIISRGVTNYADSVKGRFTISGDPAKNTAYLQMNSLKPEDTAVYYCNAHISTGWGRPHNNYWGQGTQVTVSS

SEQ ID NO: 46 - protein, 121 aa, Artificial Sequence
  Nanobody Sequence
EVQLVESGGDLVQPGGSLGLSCAASGSIFSINDMGWFRQAPGKQRELVADIISRGVTNYADSVKGRFTISGDPAKNTVYLQMNSLKPEDTAVYYCNAHISTGWGRPHNNYWGQGTQVTVSS

SEQ ID NO: 47 - protein, 121 aa, Artificial Sequence
  Nanobody Sequence
EVQLVESGGDLVRPGGSLRLSCAASGSIFSINDMGWFRQAPGKQRELVADIISRGVTNYADSVKGRFTISGDPAKNTVYLQMNSLKPEDTAVYYCNAHISTGWGRPHNNYWGQGTQVTVSS

SEQ ID NO: 48 - protein, 121 aa, Artificial Sequence
  Nanobody Sequence
EVQLVESGGDLVQPGGSLRLSCAASGSIFSINDMGWFRQAPGKQRELVADIISRGVTNCADSVKGRFTISGDPAKNTVYLQMNSLKPEDTAVYYCNAHISTGWGRPHNNYWGQGTQVTVSS

SEQ ID NO: 49 - protein, 121 aa, Artificial Sequence
  Nanobody Sequence
EVQLVESGGDLVQPGGSLRLSCAASGSIFSINDMGWLRQAPGKQRELVADIISRGVTNYADSVKGRFTISGDPAKNTVYLQMNSLKPEDTAVYYCNAHISTGWGRPHNNYWGQGTQVTVSS

SEQ ID NO: 50 - protein, 121 aa, Artificial Sequence
  Nanobody Sequence
EVQLVESGGDLVQPGGSLRLSCAASGSIFSINDMGWFRQAPGKQRELVADIISRGVTNYADSVRGRFTISGDPAKNTVYLQMNSLKPEDTAVYYCNAHISTGWGRPHNNYWGQGTQVTVSS

SEQ ID NO: 51 - protein, 121 aa, Artificial Sequence
  Nanobody Sequence
EVQLVESGGGLVQPGGSLRLSCAASGSIFSINDMGWFRQAPGKQRELVADIISRGVTNYADSVKGRFTISGDPAKNTVYLQMNSLKPEDTAVYYCNAHISTGWGRPHNNYWGQGTQVTVSS

SEQ ID NO: 52 - protein, 121 aa, Artificial Sequence
  Nanobody Sequence
EVQLVESGGDLVQPGGSLRLSCAASGSIFSINDMGWFRQAPGKQRELVADIISRGVTNYADSVKGRFTVSGDPAKNTVYLQMNSLKPEDTAVYYCNAHISTGWGRPHNNYWGQGTQVTVSS

SEQ ID NO: 53 - protein, 121 aa, Artificial Sequence
  Nanobody Sequence
EVQLVESGGDLVQPGGSLRLSCAASGSIFSINDMGWFRQAPGKQRELVADIISRGVTNYADSVKGRFTISGDHAKNTVYLQMNSLKPEDTAVYYCNAHISTGWGRPHNNYWGQGTQVTVSS

SEQ ID NO: 54 - protein, 121 aa, Artificial Sequence
  Nanobody Sequence
EVQLVESGGDLVQPGGSLRLSCAASGSIFSINDMGWFRQAPGKQRELVADIISRDVTNYADSVKGRFTISGDHAKNTVYLQMNSLKPEDTAVYYCNAHISTGWGRPHNNYWGQGTQVTVSS

SEQ ID NO: 55 - protein, 121 aa, Artificial Sequence
  Nanobody Sequence
EVQLVESGGDLVQPGGSLRLSCAASGSIFSINDMGWFRQAPGKQRELVADIISRGVTNYADSVKGRFTISGDPAKNTVYLQMNSLKPEDTAVYYCNAHISMGWGRPHNNYWGQGTLVTVSS

SEQ ID NO: 56 - protein, 115 aa, Artificial Sequence
  Nanobody Sequence
EVQLVESGGGLVQAGGSLRLSCTGSRSIFSTYAMAWHRQAPGKQRELVGFIYWGGTTTYSDSVKGRFTISRDNAKNTMYLQMNSLKPEDAGVYYCNIYGSYALPWGQGTLVTVSS

SEQ ID NO: 57 - protein, 115 aa, Artificial Sequence
  Nanobody Sequence
EVQLVESGGGLVQAGGSLRLSCTGSRNIFSTYAMAWHRQAPGKQRELVGFIYWGGTTSYVDSVKGRFTISRDNAKNTMYLQMNSLKPEDAAVYYCNIYGSYALPWGQGTLVTVSS

SEQ ID NO: 58 - protein, 115 aa, Artificial Sequence
  Nanobody Sequence
EVQLVESGGGLVQAGGSLRLSCTGSRSIFSTYAMAWHRQAPGKQRELVGFIYWGGTTTYSDSVKGRFTISRDNAKNTMYLQMNSLKPEDAGVYYCNIYGSYALPQGQGTLVTVSS

SEQ ID NO: 59 - protein, 115 aa, Artificial Sequence
  Nanobody Sequence
EVQLVESGGGMVQAGGSLRLSCTGSRNIFSTYAMAWHRQAPGKQRELVGFIYWGGTTSYVDSVKGRFTISRDNAKNTMYLQMNSLKPEDAAVYYCNIYGSYALPWGQGTQVTVSS

SEQ ID NO: 60 - protein, 115 aa, Artificial Sequence
  Nanobody Sequence
EVQLVESGGGLVQAGGSLRLSCTGSRSIFSTYAMAWHRQAPGKQRELVGFIYWGGTTSYVDSVKGRFTISRDNAKNTMYLQMNSLKPEDAAVYYCNIYGSYALPWGQGTLVTVSS

SEQ ID NO: 61 - protein, 115 aa, Artificial Sequence
  Nanobody Sequence
EVQLVESGGGLVQAGGSLRLSCTGSRSIFSTYAMAWHRQAPGKQRELVGFIYWGGTTTYSDSVKGRFTISRDNAKSTMYLQMNSLKPEDAGVYYCNIYGSYALPWGQGTLVTVSS

SEQ ID NO: 62 - protein, 120 aa, Artificial Sequence
  Nanobody Sequence
EVQLVESGGGLVQPGGSLRLSCAASGTIFSISTMGWYRQAPGKQREVVAVTSGFSTNYSSAVKGRFTLSRDPAKNTVFLQMNSLQPEDTATYYCNAYLSLAWRDPDRDYWGQGTQVTVSS

SEQ ID NO: 63 - protein, 119 aa, Artificial Sequence
  Nanobody Sequence
EVQLVESGGGLVQAGESLRLSCAASGSIFSIDAMGWYRQAPGKQRELVAEISDHTTYGDSVKGRFTISRGNAENTVALQMNSLKPEDTGVYYCNVHHQRGWGTSITVTWGQGTQVTVSS

SEQ ID NO: 64 - protein, 119 aa, Artificial Sequence
  Nanobody Sequence
EVQLVESGGGLVQAGESLRLSCAASGSIFSIDAMGWYRQAPGKQRELVAEISDHTTYGDSVKGRFTISRGNAENTVALQMNSLKPEDTGVYYCNVHHQRGWGTSITVAWGQGTQVTVSS

SEQ ID NO: 65 - protein, 119 aa, Artificial Sequence
  Nanobody Sequence
EVQLVESGGGLVQAGESLRLSCAASGSIFSIDAMGWYRQAPGKQRELVAEISDHTTYGDSMKGRFTISRGNAENTVALQMNSLKPEDTGVYYCNVHHQRGWGTSITVTWGQGTQVTVSS

SEQ ID NO: 66 - protein, 119 aa, Artificial Sequence
  Nanobody Sequence
EVQLVESGGRLVQAGESLRLSCAASGSIFSIDAMGWYRQAPGKQRELVAEISGHTTYGDSVKGRFTISRGNAENTVALQMNSLKPEDTGVYYCNVHHQRGWGTPITVTWGQGTQVTVSS

SEQ ID NO: 67 - protein, 119 aa, Artificial Sequence
  Nanobody Sequence
EVQLVESGGRLVQAGESLRLSCAASGSIFSIDAMGWYRQAPGKQRELVAEISDHTTYGDSVKGRFTISRGNAENTVALQMNSLKPEDTGVYYCNVHHQRGWGTPITVTWGQGTQVTVSS

SEQ ID NO: 68 - protein, 119 aa, Artificial Sequence
  Nanobody Sequence
EVQLVESGGGLVRAGESLRLSCAASGSIFSIDAMGWYRQAPGKQRELVAEISDHTTYGDSVKGRFTISRGNAENTVALQMNSLKPEDTGVYYCNVHHQRGWGTSITVTWGQGTLVTVSS

SEQ ID NO: 69 - protein, 115 aa, Artificial Sequence
  Nanobody Sequence
EVQLVESGGGLVQAGGSLRLSCVASGSISSITAMGWHRQAPGAQREGVAVISRSGATMLVDSVKGRFTIVQDNAKNTVYLQMNSLKVEDTAVYGCSAITQGRTYWGQGTLVTVSS

SEQ ID NO: 70 - protein, 115 aa, Artificial Sequence
  Nanobody Sequence
EVQLVESGGGLVQAGGSLRLSCVASGSISSITAMGWHRQAPGAQREGVAIISRSGATMLVDSVKGRFTIVQDNAKNTVYLQMNSLKVEDTAVYGCSAITQGRTYWGQGTQVTVSS

SEQ ID NO: 71 - protein, 115 aa, Artificial Sequence
  Nanobody Sequence
EVQLVESGGGLVQAGGSLRLSCVASGSISSITAMGWHRQAPGAQREGVAAISRSGATILADSVKGRFTIVQDNAKNTVYLQMNSLKVEDTAVYGCSAITQEQTYWGQGTQVTVSS

SEQ ID NO: 72 - protein, 118 aa, Artificial Sequence
  Nanobody Sequence
EVQLVESGGGLVQAGGSLRLSCAASGSIFSFIVMGWYRQAPGEQRALVATVTSGGDTFYVDSVKDRFTISRDNAKNTVYLQMNSLKPEDTAVYFCYFTKVSPYKETTWGQGTLVTVSS

SEQ ID NO: 73 - protein, 10 aa, Artificial Sequence
  CDR1
ETIFSIDSMA

SEQ ID NO: 74 - protein, 10 aa, Artificial Sequence
  CDR1
ESIFSIDAMG

SEQ ID NO: 75 - protein, 10 aa, Artificial Sequence
  CDR1
ESIFSINAMG

SEQ ID NO: 76 - protein, 10 aa, Artificial Sequence
  CDR1
GSIFSIDSMG

SEQ ID NO: 77 - protein, 10 aa, Artificial Sequence
  CDR1
GSIFSIDAMG

SEQ ID NO: 78 - protein, 10 aa, Artificial Sequence
  CDR1
GSIFSINAMG

SEQ ID NO: 79 - protein, 10 aa, Artificial Sequence
  CDR1
GSVFSINDMG

SEQ ID NO: 80 - protein, 10 aa, Artificial Sequence
  CDR1
GSIFSIDDMG

SEQ ID NO: 81 - protein, 10 aa, Artificial Sequence
  CDR1
GSIFSINDVG

SEQ ID NO: 82 - protein, 10 aa, Artificial Sequence
  CDR1
GNIFSINDMG

SEQ ID NO: 83 - protein, 10 aa, Artificial Sequence
  CDR1
GSIFSINDMG

SEQ ID NO: 84 - protein, 10 aa, Artificial Sequence
  CDR1
GSIFSINDTG

SEQ ID NO: 85 - protein, 10 aa, Artificial Sequence
  CDR1
RSIFSTYAMA

SEQ ID NO: 86 - protein, 10 aa, Artificial Sequence
  CDR1
RNIFSTYAMA

SEQ ID NO: 87 - protein, 10 aa, Artificial Sequence
  CDR1
GTIFSISTMG

SEQ ID NO: 88 - protein, 10 aa, Artificial Sequence
  CDR1
GSISSITAMG

SEQ ID NO: 89 - protein, 10 aa, Artificial Sequence
  CDR1
GSIFSFIVMG

SEQ ID NO: 90 - protein, 9 aa, Artificial Sequence
  CDR2
AITGGGSPN

SEQ ID NO: 91 - protein, 9 aa, Artificial Sequence
  CDR2
HITGGGRSN

SEQ ID NO: 92 - protein, 9 aa, Artificial Sequence
  CDR2
TITGGGSTN

SEQ ID NO: 93 - protein, 9 aa, Artificial Sequence
  CDR2
TITGGGRRN

SEQ ID NO: 94 - protein, 9 aa, Artificial Sequence
  CDR2
TMTGGGSTN

SEQ ID NO: 95 - protein, 9 aa, Artificial Sequence
  CDR2
HITGGGGSN

SEQ ID NO: 96 - protein, 9 aa, Artificial Sequence
  CDR2
TITGGSSTN

SEQ ID NO: 97 - protein, 9 aa, Artificial Sequence
  CDR2
HITGGGRPN

SEQ ID NO: 98 - protein, 9 aa, Artificial Sequence
  CDR2
GISGGGRTN

SEQ ID NO: 99 - protein, 9 aa, Artificial Sequence
  CDR2
AITSSTNYA

SEQ ID NO: 100 - protein, 9 aa, Artificial Sequence
  CDR2
SITSTTNYA

SEQ ID NO: 101 - protein, 9 aa, Artificial Sequence
  CDR2
AITSGTNYA

SEQ ID NO: 102 - protein, 9 aa, Artificial Sequence
  CDR2
AITSRTIYA

SEQ ID NO: 103 - protein, 9 aa, Artificial Sequence
  CDR2
TITSGKNYA

SEQ ID NO: 104 - protein, 9 aa, Artificial Sequence
  CDR2
DIISRGVTN

SEQ ID NO: 105 - protein, 9 aa, Artificial Sequence
  CDR2
DIISADVTN

SEQ ID NO: 106 - protein, 9 aa, Artificial Sequence
  CDR2
DIISAGVTN

SEQ ID NO: 107 - protein, 9 aa, Artificial Sequence
  CDR2
GIISRGVTN

SEQ ID NO: 108 - protein, 9 aa, Artificial Sequence
  CDR2
DIISRDVTN

SEQ ID NO: 109 - protein, 9 aa, Artificial Sequence
  CDR2
FIYWGGTTT

SEQ ID NO: 110 - protein, 9 aa, Artificial Sequence
  CDR2
FIYWGGTTS

SEQ ID NO: 111 - protein, 9 aa, Artificial Sequence
  CDR2
VTSGFSTNY

SEQ ID NO: 112 - protein, 9 aa, Artificial Sequence
  CDR2
EISDHTTYG

SEQ ID NO: 113 - protein, 9 aa, Artificial Sequence
  CDR2
EISGHTTYG

SEQ ID NO: 114 - protein, 9 aa, Artificial Sequence
  CDR2
VISRSGATM

SEQ ID NO: 115 - protein, 9 aa, Artificial Sequence
  CDR2
IISRSGATM

SEQ ID NO: 116 - protein, 9 aa, Artificial Sequence
  CDR2
AISRSGATI

SEQ ID NO: 117 - protein, 9 aa, Artificial Sequence
  CDR2
TVTSGGDTF

SEQ ID NO: 118 - protein, 13 aa, Artificial Sequence
  CDR3
EGQAGWGTALMDY

SEQ ID NO: 119 - protein, 13 aa, Artificial Sequence
  CDR3
EGQAGWGTPLMNY

SEQ ID NO: 120 - protein, 13 aa, Artificial Sequence
  CDR3
EGQAGWGTALINY

SEQ ID NO: 121 - protein, 13 aa, Artificial Sequence
  CDR3
KGQTGWGTALMDY

SEQ ID NO: 122 - protein, 13 aa, Artificial Sequence
  CDR3
EGQTGWGTALMDY

SEQ ID NO: 123 - protein, 13 aa, Artificial Sequence
  CDR3
EGQAGWGTALLDY

SEQ ID NO: 124 - protein, 13 aa, Artificial Sequence
  CDR3
HISTGWGRPHNNY

SEQ ID NO: 125 - protein, 13 aa, Artificial Sequence
  CDR3
HISMGWGRPHNNY

SEQ ID NO: 126 - protein, 7 aa, Artificial Sequence
  CDR3
YGSYALP

SEQ ID NO: 127 - protein, 13 aa, Artificial Sequence
  CDR3
YLSLAWRDPDRDY

SEQ ID NO: 128 - protein, 13 aa, Artificial Sequence
  CDR3
HHQRGWGTSITVT

SEQ ID NO: 129 - protein, 13 aa, Artificial Sequence
  CDR3
HHQRGWGTSITVA

SEQ ID NO: 130 - protein, 13 aa, Artificial Sequence
  CDR3
HHQRGWGTPITVT

SEQ ID NO: 131 - protein, 7 aa, Artificial Sequence
  CDR3
ITQGRTY

SEQ ID NO: 132 - protein, 7 aa, Artificial Sequence
  CDR3
ITQEQTY

SEQ ID NO: 133 - protein, 10 aa, Artificial Sequence
  CDR3
TKVSPYKETT

SEQ ID NO: 134 - protein, 25 aa, Artificial Sequence [sequence omitted]

SEQ ID NO: 135 - protein, 25 aa, Artificial Sequence
  FW1
EVQLVESGGGLVQPGGSLRLSCTAS

SEQ ID NO: 136 - protein, 25 aa, Artificial Sequence
  FW1
EVQLVESGGGLVQSGGSLRLSCAAS

SEQ ID NO: 137 - protein, 25 aa, Artificial Sequence
  FW1
EVQLVESGGGLVRPGGSLRLSCAAS

SEQ ID NO: 138 - protein, 25 aa, Artificial Sequence
  FW1
EVQLVESGGGLVRPGGSLRLPCAAS

SEQ ID NO: 139 - protein, 25 aa, Artificial Sequence
  FW1
EVQLVESGGGLVQPGGSLRLSCAGS

SEQ ID NO: 140 - protein, 25 aa, Artificial Sequence
  FW1
EVQLVESGGGLVQPGGSLRLTCAAS

SEQ ID NO: 141 - protein, 25 aa, Artificial Sequence
  FW1
EVQLVESGGGLVQPGGSLRLFCAAS

SEQ ID NO: 142 - protein, 25 aa, Artificial Sequence
  FW1
EVQLVESGGDLVQPGGSLRLSCAAS

SEQ ID NO: 143 - protein, 25 aa, Artificial Sequence
  FW1
EVQLVESGGDLVQPGGPLRLSCAAS

SEQ ID NO: 144 - protein, 25 aa, Artificial Sequence
  FW1
EVQLVESGGDLVQPGGSLGLSCAAS

SEQ ID NO: 145 - protein, 25 aa, Artificial Sequence
  FW1
EVQLVESGGDLVRPGGSLRLSCAAS

SEQ ID NO: 146 - protein, 25 aa, Artificial Sequence
  FW1
EVQLVESGGGLVQAGGSLRLSCTGS

SEQ ID NO: 147 - protein, 25 aa, Artificial Sequence
  FW1
EVQLVESGGGMVQAGGSLRLSCTGS

SEQ ID NO: 148 - protein, 25 aa, Artificial Sequence
  FW1
EVQLVESGGGLVQAGESLRLSCAAS

SEQ ID NO: 149 - protein, 25 aa, Artificial Sequence
  FW1
EVQLVESGGRLVQAGESLRLSCAAS

SEQ ID NO: 150 - protein, 25 aa, Artificial Sequence
  FW1
EVQLVESGGGLVRAGESLRLSCAAS

SEQ ID NO: 151 - protein, 25 aa, Artificial Sequence
  FW1
EVQLVESGGGLVQAGGSLRLSCVAS

SEQ ID NO: 152 - protein, 25 aa, Artificial Sequence
  FW1
EVQLVESGGGLVQAGGSLRLSCAAS

SEQ ID NO: 153 - protein, 14 aa, Artificial Sequence
  FW2
WYRQAPGKQRELVA

SEQ ID NO: 154 - protein, 14 aa, Artificial Sequence
  FW2
WHRQAPGKQRELVA

SEQ ID NO: 155 - protein, 14 aa, Artificial Sequence
  FW2
WYHQAPGKQRELVA

SEQ ID NO: 156 - protein, 14 aa, Artificial Sequence
  FW2
WYRQAPGRQRELVA

SEQ ID NO: 157 - protein, 14 aa, Artificial Sequence
  FW2
WFRQAPGKQRELVA

SEQ ID NO: 158 - protein, 14 aa, Artificial Sequence
  FW2
WLRQAPGKQRELVA

SEQ ID NO: 159 - protein, 14 aa, Artificial Sequence
  FW2
WHRQAPGKQRELVG

SEQ ID NO: 160 - protein, 14 aa, Artificial Sequence
  FW2
WYRQAPGKQREVVA

SEQ ID NO: 161 - protein, 14 aa, Artificial Sequence
  FW2
WHRQAPGAQREGVA

SEQ ID NO: 162 - protein, 14 aa, Artificial Sequence
  FW2
WYRQAPGEQRALVA

SEQ ID NO: 163 - protein, 39 aa, Artificial Sequence
  FW3
YADSVKGRFTISSDVAKRTVYLQMNSLKPEDTAVYYCNA

SEQ ID NO: 164 - protein, 39 aa, Artificial Sequence
  FW3
YADSVKGRFTISGDSAKRTVYLQMNSLKPEDTAVYYCNA

SEQ ID NO: 165 - protein, 39 aa, Artificial Sequence
  FW3
YADSVKGRFTISGDSAKRTVYLQMDSLKPEDTAVYYCNA

SEQ ID NO: 166 - protein, 39 aa, Artificial Sequence
  FW3
YADSVMGRFSISGDNAKRTVYLQMNSLKPEDTAVYYCNA

SEQ ID NO: 167 - protein, 39 aa, Artificial Sequence
  FW3
YADSVKGRFTISGDSAKRTVYLQMNSLRPEDTAVYYCNA

SEQ ID NO: 168 - protein, 39 aa, Artificial Sequence
  FW3
YADSVKGRFTISSDVAKRTAYLQMNSLKPEDTAVYYCNA

SEQ ID NO: 169 - protein, 39 aa, Artificial Sequence
  FW3
YADSVRGRFTISSDVAKRTVYLQMNSLKPEDTAVYYCNA

SEQ ID NO: 170 - protein, 39 aa, Artificial Sequence
  FW3
YADSVKGRFAISGDSAKRTVYLQMNSLKPEDTAVYYCNA

SEQ ID NO: 171 - protein, 39 aa, Artificial Sequence
  FW3
YADSVKGRFTISGDNAKRTVYLQMNSLKPEDTAVYYCNA

SEQ ID NO: 172 - protein, 39 aa, Artificial Sequence
  FW3
YADSVKGRFTISGDNAKRTVYLQMNSLKPEDTAAYYCNA

SEQ ID NO: 173 - protein, 39 aa, Artificial Sequence
  FW3
YADSVKGRFTISGDSAKRTVYLQMNSLKPGDTAVYYCNA

SEQ ID NO: 174 - protein, 39 aa, Artificial Sequence
  FW3
YADSVKGRFTISGDNAKNTVYLQMNSLKPEDTAVYYCNA

SEQ ID NO: 175 - protein, 37 aa, Artificial Sequence
  FW3
DSVKGRFTISRDNAKNTVYLQMNSLKPEDTAVYYCNL

SEQ ID NO: 176 - protein, 37 aa, Artificial Sequence
  FW3
ESVKGRFTISRANAKNTVYLQMNSLKPEDTAVYYCNV

SEQ ID NO: 177 - protein, 37 aa, Artificial Sequence
  FW3
ESVKGRFTISRANAKNTVYLQMNSLKPEDTAVYYCSV

SEQ ID NO: 178 - protein, 37 aa, Artificial Sequence
  FW3
DSAKGRFTISRDHAKNTVYLQMNSLKPEDTAVYYCNL

SEQ ID NO: 179 - protein, 37 aa, Artificial Sequence
  FW3
DSVKGRFTISRDHAKNTVYLQMNSLKPEDTAVYYCNL

SEQ ID NO: 180 - protein, 37 aa, Artificial Sequence
  FW3
DSVRGRFTISRDHAKNTVYLQMNSLKPEDTAVYYCNL

SEQ ID NO: 181 - protein, 37 aa, Artificial Sequence
  FW3
DSVKGRFTISRDNAKNAVYLQMNSLKPEDTAVYYCNL

SEQ ID NO: 182 - protein, 37 aa, Artificial Sequence
  FW3
DSVKGRFTISRDNAKNTVYLQTNSLKPEDTAVYYCNL

SEQ ID NO: 183 - protein, 37 aa, Artificial Sequence
  FW3
DSVKGRFTISRANAKNTVYLQMNSLKPEDTAVYYCHL

SEQ ID NO: 184 - protein, 39 aa, Artificial Sequence
  FW3
YADSVKGRFTISGDPAKNTVYLQMNSLKPEDTAVYYCNA

SEQ ID NO: 185 - protein, 39 aa, Artificial Sequence
  FW3
YADSVKGRFTISGDHAKNTVYLQMNSLKPEDTAVYYCNA

SEQ ID NO: 186 - protein, 39 aa, Artificial Sequence
  FW3
YADSVKGRFTISGDHAQNTVYLQMNSLKPEDTAVYYCNA

SEQ ID NO: 187 - protein, 39 aa, Artificial Sequence
  FW3
YADSVKGRFTISGDPAKNTVYLQMNSLKPEDTAAYYCNA

SEQ ID NO: 188 - protein, 39 aa, Artificial Sequence
  FW3
YADSVKGRFTISGDPAKNTAYLQMNSLKPEDTAVYYCNA

SEQ ID NO: 189 - protein, 39 aa, Artificial Sequence
  FW3
CADSVKGRFTISGDPAKNTVYLQMNSLKPEDTAVYYCNA

SEQ ID NO: 190 - protein, 39 aa, Artificial Sequence
  FW3
YADSVRGRFTISGDPAKNTVYLQMNSLKPEDTAVYYCNA

SEQ ID NO: 191 - protein, 39 aa, Artificial Sequence
  FW3
YADSVKGRFTVSGDPAKNTVYLQMNSLKPEDTAVYYCNA

SEQ ID NO: 192 - protein, 39 aa, Artificial Sequence
  FW3
YSDSVKGRFTISRDNAKNTMYLQMNSLKPEDAGVYYCNI

SEQ ID NO: 193 - protein, 39 aa, Artificial Sequence
  FW3
YVDSVKGRFTISRDNAKNTMYLQMNSLKPEDAAVYYCNI

SEQ ID NO: 194 - protein, 39 aa, Artificial Sequence
  FW3
YSDSVKGRFTISRDNAKSTMYLQMNSLKPEDAGVYYCNI

SEQ ID NO: 195 - protein, 38 aa, Artificial Sequence
  FW3
SSAVKGRFTLSRDPAKNTVFLQMNSLQPEDTATYYCNA

SEQ ID NO: 196 - protein, 37 aa, Artificial Sequence
  FW3
DSVKGRFTISRGNAENTVALQMNSLKPEDTGVYYCNV

SEQ ID NO: 197 - protein, 37 aa, Artificial Sequence
  FW3
DSMKGRFTISRGNAENTVALQMNSLKPEDTGVYYCNV

SEQ ID NO: 198 - protein, 39 aa, Artificial Sequence
  FW3
LVDSVKGRFTIVQDNAKNTVYLQMNSLKVEDTAVYGCSA

SEQ ID NO: 199 - protein, 39 aa, Artificial Sequence
  FW3
LADSVKGRFTIVQDNAKNTVYLQMNSLKVEDTAVYGCSA

SEQ ID NO: 200 - protein, 39 aa, Artificial Sequence
  FW3
YVDSVKDRFTISRDNAKNTVYLQMNSLKPEDTAVYFCYF

SEQ ID NO: 201 - protein, 11 aa, Artificial Sequence
  FW4
WGKGTLVTVSS

SEQ ID NO: 202 - protein, 11 aa, Artificial Sequence
  FW4
WGKGTQVTVSS

SEQ ID NO: 203 - protein, 11 aa, Artificial Sequence
  FW4
WGQGTQVTVSS

SEQ ID NO: 204 - protein, 11 aa, Artificial Sequence
  FW4
WGQGTLVTVSS

SEQ ID NO: 205 - protein, 11 aa, Artificial Sequence
  FW4
QGQGTLVTVSS

SEQ ID NO: 206 - protein, 423 aa, Artificial Sequence
  Nanobody Sequence
EVQLVESGGGLVQPGGSLRLSCAASGSIFSIDSMGWYRQAPGKQRELVAAITSSTNYADSVKGRFTISRDNAKNTVYLQMNSLKPEDTAVYYCNLEGQAGWGTALINYWGKGTLVTVSSGGGGSGGGGSGGGGSGGGGSGGGGSGGGGSGGGGSEVQLVESGGGLVQPGGSLRLSCAASGSIFSIDSMGWYRQAPGKQRELVAAITSSTNYADSVKGRFTISRDNAKNTVYLQMNSLKPEDTAVYYCNLEGQAGWGTALINYWGKGTLVTVSSGGGGSGGGGSGGGGSGGGGSGGGGSGGGGSGGGGSEVQLVESGGGLVQPGNSLRLSCAASGFTFSSFGMSWVRQAPGKGLEWVSSISGSGSDTLYADSVKGRFTISRDNAKTTLYLQMNSLRPEDTAVYYCTIGGSLSRSSQGTLVTVSS

SEQ ID NO: 207 - protein, 427 aa, Artificial Sequence
  Nanobody Sequence
EVQLVESGGGLVQPGGSLRLSCAASETIFSIDSMAWYRQAPGKQRELVAAITGGGSPNYADSVKGRFTISSDVAKRTVYLQMNSLKPEDTAVYYCNAEGQAGWGTALMDYWGKGTLVTVSSGGGGSGGGGSGGGGSGGGGSGGGGSGGGGSGGGGSEVQLVESGGGLVQPGGSLRLSCAASETIFSIDSMAWYRQAPGKQRELVAAITGGGSPNYADSVKGRFTISSDVAKRTVYLQMNSLKPEDTAVYYCNAEGQAGWGTALMDYWGKGTLVTVSSGGGGSGGGGSGGGGSGGGGSGGGGSGGGGSGGGGSEVQLVESGGGLVQPGNSLRLSCAASGFTFSSFGMSWVRQAPGKGLEWVSSISGSGSDTLYADSVKGRFTISRDNAKTTLYLQMNSLRPEDTAVYYCTIGGSLSRSSQGTLVTVSS

SEQ ID NO: 208 - protein, 415 aa, Artificial Sequence
  Nanobody Sequence
EVQLVESGGGLVQAGGSLRLSCVASGSISSITAMGWHRQAPGAQREGVAVISRSGATMLVDSVKGRFTIVQDNAKNTVYLQMNSLKVEDTAVYGCSAITQGRTYWGQGTLVTVSSGGGGSGGGGSGGGGSGGGGSGGGGSGGGGSGGGGSEVQLVESGGGLVQAGGSLRLSCVASGSISSITAMGWHRQAPGAQREGVAVISRSGATMLVDSVKGRFTIVQDNAKNTVYLQMNSLKVEDTAVYGCSAITQGRTYWGQGTLVTVSSGGGGSGGGGSGGGGSGGGGSGGGGSGGGGSGGGGSEVQLVESGGGLVQPGNSLRLSCAASGFTFSSFGMSWVRQAPGKGLEWVSSISGSGSDTLYADSVKGRFTISRDNAKTTLYLQMNSLRPEDTAVYYCTIGGSLSRSSQGTLVTVSS

SEQ ID NO: 209 - protein, 577 aa, Artificial Sequence
  Nanobody Sequence
EVQLVESGGGLVQPGGSLRLSCAASGSIFSIDSMGWYRQAPGKQRELVAAITSSTNYADSVKGRFTISRDNAKNTVYLQMNSLKPEDTAVYYCNLEGQAGWGTALINYWGKGTLVTVSSGGGGSGGGGSGGGGSGGGGSGGGGSGGGGSGGGGSEVQLVESGGGLVQPGGSLRLSCAASGSIFSIDSMGWYRQAPGKQRELVAAITSSTNYADSVKGRFTISRDNAKNTVYLQMNSLKPEDTAVYYCNLEGQAGWGTALINYWGKGTLVTVSSGGGGSGGGGSGGGGSGGGGSGGGGSGGGGSGGGGSEVQLVESGGGLVQPGGSLRLSCAASGSIFSIDSMGWYRQAPGKQRELVAAITSSTNYADSVKGRFTISRDNAKNTVYLQMNSLKPEDTAVYYCNLEGQAGWGTALINYWGKGTLVTVSSGGGGSGGGGSGGGGSGGGGSGGGGSGGGGSGGGGSEVQLVESGGGLVQPGNSLRLSCAASGFTFSSFGMSWVRQAPGKGLEWVSSISGSGSDTLYADSVKGRFTISRDNAKTTLYLQMNSLRPEDTAVYYCTIGGSLSRSSQGTLVTVSS

SEQ ID NO: 210 - protein, 565 aa, Artificial Sequence
  Nanobody Sequence
EVQLVESGGGLVQAGGSLRLSCVASGSISSITAMGWHRQAPGAQREGVAVISRSGATMLVDSVKGRFTIVQDNAKNTVYLQMNSLKVEDTAVYGCSAITQGRTYWGQGTLVTVSSGGGGSGGGGSGGGGSGGGGSGGGGSGGGGSGGGGSEVQLVESGGGLVQAGGSLRLSCVASGSISSITAMGWHRQAPGAQREGVAVISRSGATMLVDSVKGRFTIVQDNAKNTVYLQMNSLKVEDTAVYGCSAITQGRTYWGQGTLVTVSSGGGGSGGGGSGGGGSGGGGSGGGGSGGGGSGGGGSEVQLVESGGGLVQAGGSLRLSCVASGSISSITAMGWHRQAPGAQREGVAVISRSGATMLVDSVKGRFTIVQDNAKNTVYLQMNSLKVEDTAVYGCSAITQGRTYWGQGTLVTVSSGGGGSGGGGSGGGGSGGGGSGGGGSGGGGSGGGGSEVQLVESGGGLVQPGNSLRLSCAASGFTFSSFGMSWVRQAPGKGLEWVSSISGSGSDTLYADSVKGRFTISRDNAKTTLYLQMNSLRPEDTAVYYCTIGGSLSRSSQGTLVTVSS

SEQ ID NO: 211 - protein, 577 aa, Artificial Sequence
  Nanobody Sequence
EVQLVESGGGLVQAGESLRLSCAASGSIFSIDAMGWYRQAPGKQRELVAEISDHTTYGDSVKGRFTISRGNAENTVALQMNSLKPEDTGVYYCNVHHQRGWGTSITVTWGQGTLVTVSSGGGGSGGGGSGGGGSGGGGSGGGGSGGGGSGGGGSEVQLVESGGGLVQAGESLRLSCAASGSIFSIDAMGWYRQAPGKQRELVAEISDHTTYGDSVKGRFTISRGNAENTVALQMNSLKPEDTGVYYCNVHHQRGWGTSITVTWGQGTLVTVSSGGGGSGGGGSGGGGSGGGGSGGGGSGGGGSGGGGSEVQLVESGGGLVQAGESLRLSCAASGSIFSIDAMGWYRQAPGKQRELVAEISDHTTYGDSVKGRFTISRGNAENTVALQMNSLKPEDTGVYYCNVHHQRGWGTSITVTWGQGTLVTVSSGGGGSGGGGSGGGGSGGGGSGGGGSGGGGSGGGGSEVQLVESGGGLVQPGNSLRLSCAASGFTFSSFGMSWVRQAPGKGLEWVSSISGSGSDTLYADSVKGRFTISRDNAKTTLYLQMNSLRPEDTAVYYCTIGGSLSRSSQGTLVTVSS

SEQ ID NO: 212 - protein, 583 aa, Artificial Sequence
  Nanobody Sequence
EVQLVESGGGLVQPGGSLRLSCAASETIFSIDSMAWYRQAPGKQRELVAAITGGGSPNYADSVKGRFTISSDVAKRTVYLQMNSLKPEDTAVYYCNAEGQAGWGTALMDYWGKGTLVTVSSGGGGSGGGGSGGGGSGGGGSGGGGSGGGGSGGGGSEVQLVESGGGLVQPGGSLRLSCAASETIFSIDSMAWYRQAPGKQRELVAAITGGGSPNYADSVKGRFTISSDVAKRTVYLQMNSLKPEDTAVYYCNAEGQAGWGTALMDYWGKGTLVTVSSGGGGSGGGGSGGGGSGGGGSGGGGSGGGGSGGGGSEVQLVESGGGLVQPGGSLRLSCAASETIFSIDSMAWYRQAPGKQRELVAAITGGGSPNYADSVKGRFTISSDVAKRTVYLQMNSLKPEDTAVYYCNAEGQAGWGTALMDYWGKGTLVTVSSGGGGSGGGGSGGGGSGGGGSGGGGSGGGGSGGGGSEVQLVESGGGLVQPGNSLRLSCAASGFTFSSFGMSWVRQAPGKGLEWVSSISGSGSDTLYADSVKGRFTISRDNAKTTLYLQMNSLRPEDTAVYYCTIGGSLSRSSQGTLVTVSS

SEQ ID NO: 213 - protein, 565 aa, Artificial Sequence
  Nanobody Sequence
EVQLVESGGGLVQAGGSLRLSCTGSRSIFSTYAMAWHRQAPGKQRELVGFIYWGGTTTYSDSVKGRFTISRDNAKNTMYLQMNSLKPEDAGVYYCNIYGSYALPWGQGTLVTVSSGGGGSGGGGSGGGGSGGGGSGGGGSGGGGSGGGGSEVQLVESGGGLVQAGGSLRLSCTGSRSIFSTYAMAWHRQAPGKQRELVGFIYWGGTTTYSDSVKGRFTISRDNAKNTMYLQMNSLKPEDAGVYYCNIYGSYALPWGQGTLVTVSSGGGGSGGGGSGGGGSGGGGSGGGGSGGGGSGGGGSEVQLVESGGGLVQAGGSLRLSCTGSRSIFSTYAMAWHRQAPGKQRELVGFIYWGGTTTYSDSVKGRFTISRDNAKNTMYLQMNSLKPEDAGVYYCNIYGSYALPWGQGTLVTVSSGGGGSGGGGSGGGGSGGGGSGGGGSGGGGSGGGGSEVQLVESGGGLVQPGNSLRLSCAASGFTFSSFGMSWVRQAPGKGLEWVSSISGSGSDTLYADSVKGRFTISRDNAKTTLYLQMNSLRPEDTAVYYCTIGGSLSRSSQGTLVTVSS

SEQ ID NO: 214 - protein, 583 aa, Artificial Sequence
  Nanobody Sequence
EVQLVESGGDLVQPGGSLRLSCAASGSVFSINDMGWFRQAPGKQRELVADIISRGVTNYADSVKGRFTISGDPAKNTVYLQMNSLKPEDTAVYYCNAHISTGWGRPHNNYWGQGTLVTVSSGGGGSGGGGSGGGGSGGGGSGGGGSGGGGSGGGGSEVQLVESGGDLVQPGGSLRLSCAASGSVFSINDMGWFRQAPGKQRELVADIISRGVTNYADSVKGRFTISGDPAKNTVYLQMNSLKPEDTAVYYCNAHISTGWGRPHNNYWGQGTLVTVSSGGGGSGGGGSGGGGSGGGGSGGGGSGGGGSGGGGSEVQLVESGGDLVQPGGSLRLSCAASGSVFSINDMGWFRQAPGKQRELVADIISRGVTNYADSVKGRFTISGDPAKNTVYLQMNSLKPEDTAVYYCNAHISTGWGRPHNNYWGQGTLVTVSSGGGGSGGGGSGGGGSGGGGSGGGGSGGGGSGGGGSEVQLVESGGGLVQPGNSLRLSCAASGFTFSSFGMSWVRQAPGKGLEWVSSISGSGSDTLYADSVKGRFTISRDNAKTTLYLQMNSLRPEDTAVYYCTIGGSLSRSSQGTLVTVSS

SEQ ID NO: 215 - protein, 580 aa, Artificial Sequence
  Nanobody Sequence
EVQLVESGGGLVQPGGSLRLSCAASGTIFSISTMGWYRQAPGKQREVVAVTSGFSTNYSSAVKGRFTLSRDPAKNTVFLQMNSLQPEDTATYYCNAYLSLAWRDPDRDYWGQGTLVTVSSGGGGSGGGGSGGGGSGGGGSGGGGSGGGGSGGGGSEVQLVESGGGLVQPGGSLRLSCAASGTIFSISTMGWYRQAPGKQREVVAVTSGFSTNYSSAVKGRFTLSRDPAKNTVFLQMNSLQPEDTATYYCNAYLSLAWRDPDRDYWGQGTLVTVSSGGGGSGGGGSGGGGSGGGGSGGGGSGGGGSGGGGSEVQLVESGGGLVQPGGSLRLSCAASGTIFSISTMGWYRQAPGKQREVVAVTSGFSTNYSSAVKGRFTLSRDPAKNTVFLQMNSLQPEDTATYYCNAYLSLAWRDPDRDYWGQGTLVTVSSGGGGSGGGGSGGGGSGGGGSGGGGSGGGGSGGGGSEVQLVESGGGLVQPGNSLRLSCAASGFTFSSFGMSWVRQAPGKGLEWVSSISGSGSDTLYADSVKGRFTISRDNAKTTLYLQMNSLRPEDTAVYYCTIGGSLSRSSQGTLVTVSS

SEQ ID NO: 216 - protein, 375 aa, Artificial Sequence
  Nanobody Sequence
EVQLVESGGGLVQPGGSLRLSCAASETIFSIDSMAWYRQAPGKQRELVAAITGGGSPNYADSVKGRFTISSDVAKRTVYLQMNSLKPEDTAVYYCNAEGQAGWGTALMDYWGKGTLVTVSSGGGGSGGGSEVQLVESGGGLVQPGGSLRLSCAASETIFSIDSMAWYRQAPGKQRELVAAITGGGSPNYADSVKGRFTISSDVAKRTVYLQMNSLKPEDTAVYYCNAEGQAGWGTALMDYWGKGTLVTVSSGGGGSGGGSEVQLVESGGGLVQPGNSLRLSCAASGFTFSSFGMSWVRQAPGKGLEWVSSISGSGSDTLYADSVKGRFTISRDNAKTTLYLQMNSLRPEDTAVYYCTIGGSLSRSSQGTLVTVSS

SEQ ID NO: 217 - protein, 427 aa, Artificial Sequence; identical to SEQ ID NO: 207
  Nanobody Sequence

SEQ ID NO: 218 - protein, 505 aa, Artificial Sequence
  Nanobody Sequence
EVQLVESGGGLVQPGGSLRLSCAASETIFSIDSMAWYRQAPGKQRELVAAITGGGSPNYADSVKGRFTISSDVAKRTVYLQMNSLKPEDTAVYYCNAEGQAGWGTALMDYWGKGTLVTVSSGGGGSGGGSEVQLVESGGGLVQPGGSLRLSCAASETIFSIDSMAWYRQAPGKQRELVAAITGGGSPNYADSVKGRFTISSDVAKRTVYLQMNSLKPEDTAVYYCNAEGQAGWGTALMDYWGKGTLVTVSSGGGGSGGGSEVQLVESGGGLVQPGGSLRLSCAASETIFSIDSMAWYRQAPGKQRELVAAITGGGSPNYADSVKGRFTISSDVAKRTVYLQMNSLKPEDTAVYYCNAEGQAGWGTALMDYWGKGTLVTVSSGGGGSGGGSEVQLVESGGGLVQPGNSLRLSCAASGFTFSSFGMSWVRQAPGKGLEWVSSISGSGSDTLYADSVKGRFTISRDNAKTTLYLQMNSLRPEDTAVYYCTIGGSLSRSSQGTLVTVSS

SEQ ID NO: 219 - protein, 365 aa, Artificial Sequence
  Nanobody Sequence
EVQLVESGGGLVQPGGSLRLSCAASGSIFSIDSMGWYRQAPGKQRELVAAITSSTNYADSVKGRFTISRDNAKNTVYLQMNSLKPEDTAVYYCNLEGQAGWGTALINYWGKGTLVTVSSAAAEVQLVESGGGLVQPGGSLRLSCAASGSIFSIDSMGWYRQAPGKQRELVAAITSSTNYADSVKGRFTISRDNAKNTVYLQMNSLKPEDTAVYYCNLEGQAGWGTALINYWGKGTLVTVSSGGGGSGGGSEVQLVESGGGLVQPGNSLRLSCAASGFTFSSFGMSWVRQAPGKGLEWVSSISGSGSDTLYADSVKGRFTISRDNAKTTLYLQMNSLRPEDTAVYYCTIGGSLSRSSQGTLVTVSS

SEQ ID NO: 220 - protein, 359 aa, Artificial Sequence
  Nanobody Sequence
EVQLVESGGGLVQPGGSLRLSCAASGSIFSIDSMGWYRQAPGKQRELVAAITSSTNYADSVKGRFTISRDNAKNTVYLQMNSLKPEDTAVYYCNLEGQAGWGTALINYWGKGTLVTVSSAAAEVQLVESGGGLVQPGGSLRLSCAASGSIFSIDSMGWYRQAPGKQRELVAAITSSTNYADSVKGRFTISRDNAKNTVYLQMNSLKPEDTAVYYCNLEGQAGWGTALINYWGKGTLVTVSSAAAEVQLVESGGGLVQPGNSLRLSCAASGFTFSSFGMSWVRQAPGKGLEWVSSISGSGSDTLYADSVKGRFTISRDNAKTTLYLQMNSLRPEDTAVYYCTIGGSLSRSSQGTLVTVSS

SEQ ID NO: 221 - protein, 371 aa, Artificial Sequence
  Nanobody Sequence
EVQLVESGGGLVQPGGSLRLSCAASGSIFSIDSMGWYRQAPGKQRELVAAITSSTNYADSVKGRFTISRDNAKNTVYLQMNSLKPEDTAVYYCNLEGQAGWGTALINYWGKGTLVTVSSGGGGSGGGSEVQLVESGGGLVQPGGSLRLSCAASGSIFSIDSMGWYRQAPGKQRELVAAITSSTNYADSVKGRFTISRDNAKNTVYLQMNSLKPEDTAVYYCNLEGQAGWGTALINYWGKGTLVTVSSGGGGSGGGSEVQLVESGGGLVQPGNSLRLSCAASGFTFSSFGMSWVRQAPGKGLEWVSSISGSGSDTLYADSVKGRFTISRDNAKTTLYLQMNSLRPEDTAVYYCTIGGSLSRSSQGTLVTVSS

SEQ ID NO: 222 - protein, 499 aa, Artificial Sequence
  Nanobody Sequence
EVQLVESGGGLVQPGGSLRLSCAASGSIFSIDSMGWYRQAPGKQRELVAAITSSTNYADSVKGRFTISRDNAKNTVYLQMNSLKPEDTAVYYCNLEGQAGWGTALINYWGKGTLVTVSSGGGGSGGGSEVQLVESGGGLVQPGGSLRLSCAASGSIFSIDSMGWYRQAPGKQRELVAAITSSTNYADSVKGRFTISRDNAKNTVYLQMNSLKPEDTAVYYCNLEGQAGWGTALINYWGKGTLVTVSSGGGGSGGGSEVQLVESGGGLVQPGGSLRLSCAASGSIFSIDSMGWYRQAPGKQRELVAAITSSTNYADSVKGRFTISRDNAKNTVYLQMNSLKPEDTAVYYCNLEGQAGWGTALINYWGKGTLVTVSSGGGGSGGGSEVQLVESGGGLVQPGNSLRLSCAASGFTFSSFGMSWVRQAPGKGLEWVSSISGSGSDTLYADSVKGRFTISRDNAKTTLYLQMNSLRPEDTAVYYCTIGGSLSRSSQGTLVTVSS

SEQ ID NO: 223 - protein, 481 aa, Artificial Sequence
  Nanobody Sequence
EVQLVESGGGLVQPGGSLRLSCAASGSIFSIDSMGWYRQAPGKQRELVAAITSSTNYADSVKGRFTISRDNAKNTVYLQMNSLKPEDTAVYYCNLEGQAGWGTALINYWGKGTLVTVSSAAAEVQLVESGGGLVQPGGSLRLSCAASGSIFSIDSMGWYRQAPGKQRELVAAITSSTNYADSVKGRFTISRDNAKNTVYLQMNSLKPEDTAVYYCNLEGQAGWGTALINYWGKGTLVTVSSAAAEVQLVESGGGLVQPGGSLRLSCAASGSIFSIDSMGWYRQAPGKQRELVAAITSSTNYADSVKGRFTISRDNAKNTVYLQMNSLKPEDTAVYYCNLEGQAGWGTALINYWGKGTLVTVSSAAAEVQLVESGGGLVQPGNSLRLSCAASGFTFSSFGMSWVRQAPGKGLEWVSSISGSGSDTLYADSVKGRFTISRDNAKTTLYLQMNSLRPEDTAVYYCTIGGSLSRSSQGTLVTVSS

SEQ ID NO: 224 - protein, 421 aa, Artificial Sequence
  Nanobody Sequence
EVQLVESGGGLVQAGGSLRLSCAASGSIFSFIVMGWYRQAPGEQRALVATVTSGGDTFYVDSVKDRFTISRDNAKNTVYLQMNSLKPEDTAVYFCYFTKVSPYKETTWGQGTLVTVSSGGGGSGGGGSGGGGSGGGGSGGGGSGGGGSGGGGSEVQLVESGGGLVQAGGSLRLSCAASGSIFSFIVMGWYRQAPGEQRALVATVTSGGDTFYVDSVKDRFTISRDNAKNTVYLQMNSLKPEDTAVYFCYFTKVSPYKETTWGQGTLVTVSSGGGGSGGGGSGGGGSGGGGSGGGGSGGGGSGGGGSEVQLVESGGGLVQPGNSLRLSCAASGFTFSSFGMSWVRQAPGKGLEWVSSISGSGSDTLYADSVKGRFTISRDNAKTTLYLQMNSLRPEDTAVYYCTIGGSLSRSSQGTLVTVSS

SEQ ID NO: 225 - protein, 574 aa, Artificial Sequence
  Nanobody Sequence
EVQLVESGGGLVQAGGSLRLSCAASGSIFSFIVMGWYRQAPGEQRALVATVTSGGDTFYVDSVKDRFTISRDNAKNTVYLQMNSLKPEDTAVYFCYFTKVSPYKETTWGQGTLVTVSSGGGGSGGGGSGGGGSGGGGSGGGGSGGGGSGGGGSEVQLVESGGGLVQAGGSLRLSCAASGSIFSFIVMGWYRQAPGEQRALVATVTSGGDTFYVDSVKDRFTISRDNAKNTVYLQMNSLKPEDTAVYFCYFTKVSPYKETTWGQGTLVTVSSGGGGSGGGGSGGGGSGGGGSGGGGSGGGGSGGGGSEVQLVESGGGLVQAGGSLRLSCAASGSIFSFIVMGWYRQAPGEQRALVATVTSGGDTFYVDSVKDRFTISRDNAKNTVYLQMNSLKPEDTAVYFCYFTKVSPYKETTWGQGTLVTVSSGGGGSGGGGSGGGGSGGGGSGGGGSGGGGSGGGGSEVQLVESGGGLVQPGNSLRLSCAASGFTFSSFGMSWVRQAPGKGLEWVSSISGSGSDTLYADSVKGRFTISRDNAKTTLYLQMNSLRPEDTAVYYCTIGGSLSRSSQGTLVTVSS

SEQ ID NO: 226 - protein, 369 aa, Artificial Sequence
  Nanobody Sequence
EVQLVESGGGLVQAGGSLRLSCAASGSIFSFIVMGWYRQAPGEQRALVATVTSGGDTFYVDSVKDRFTISRDNAKNTVYLQMNSLKPEDTAVYFCYFTKVSPYKETTWGQGTLVTVSSGGGGSGGGSEVQLVESGGGLVQAGGSLRLSCAASGSIFSFIVMGWYRQAPGEQRALVATVTSGGDTFYVDSVKDRFTISRDNAKNTVYLQMNSLKPEDTAVYFCYFTKVSPYKETTWGQGTLVTVSSGGGGSGGGSEVQLVESGGGLVQPGNSLRLSCAASGFTFSSFGMSWVRQAPGKGLEWVSSISGSGSDTLYADSVKGRFTISRDNAKTTLYLQMNSLRPEDTAVYYCTIGGSLSRSSQGTLVTVSS

SEQ ID NO: 227 - protein, 496 aa, Artificial Sequence
  Nanobody Sequence
EVQLVESGGGLVQAGGSLRLSCAASGSIFSFIVMGWYRQAPGEQRALVATVTSGGDTFYVDSVKDRFTISRDNAKNTVYLQMNSLKPEDTAVYFCYFTKVSPYKETTWGQGTLVTVSSGGGGSGGGSEVQLVESGGGLVQAGGSLRLSCAASGSIFSFIVMGWYRQAPGEQRALVATVTSGGDTFYVDSVKDRFTISRDNAKNTVYLQMNSLKPEDTAVYFCYFTKVSPYKETTWGQGTLVTVSSGGGGSGGGSEVQLVESGGGLVQAGGSLRLSCAASGSIFSFIVMGWYRQAPGEQRALVATVTSGGDTFYVDSVKDRFTISRDNAKNTVYLQMNSLKPEDTAVYFCYFTKVSPYKETTWGQGTLVTVSSGGGGSGGGSEVQLVESGGGLVQPGNSLRLSCAASGFTFSSFGMSWVRQAPGKGLEWVSSISGSGSDTLYADSVKGRFTISRDNAKTTLYLQMNSLRPEDTAVYYCTIGGSLSRSSQGTLVTVSS

SEQ ID NO: 228 - protein, 619 aa, Artificial Sequence
  Nanobody Sequence
EVQLVESGGGSVQAGGSLRLSCAASGYTIGPYCMGWFRQAPGKEREGVAAINMGGGITYYADSVKGRFTISQDNAKNTVYLLMNSLEPEDTAIYYCAADSTIYASYYECGHGLSTGGYGYDSWGQGTLVTVSSGGGGSGGGGSGGGGSGGGGSGGGGSGGGGSGGGGSEVQLVESGGGSVQAGGSLRLSCAASGYTIGPYCMGWFRQAPGKEREGVAAINMGGGITYYADSVKGRFTISQDNAKNTVYLLMNSLEPEDTAIYYCAADSTIYASYYECGHGLSTGGYGYDSWGQGTLVTVSSGGGGSGGGGSGGGGSGGGGSGGGGSGGGGSGGGGSEVQLVESGGGSVQAGGSLRLSCAASGYTIGPYCMGWFRQAPGKEREGVAAINMGGGITYYADSVKGRFTISQDNAKNTVYLLMNSLEPEDTAIYYCAADSTIYASYYECGHGLSTGGYGYDSWGQGTLVTVSSGGGGSGGGGSGGGGSGGGGSGGGGSGGGGSGGGGSEVQLVESGGGLVQPGNSLRLSCAASGFTFSSFGMSWVRQAPGKGLEWVSSISGSGSDTLYADSVKGRFTISRDNAKTTLYLQMNSLRPEDTAVYYCTIGGSLSRSSQGTLVTVSS

SEQ ID NO: 229 - protein, 248 aa, Artificial Sequence
  Nanobody Chimera Sequence
MSVPTQVLGLLLLWLTDARCEVQLVESGGGLVQPGGSLRLSCAASETIFSIDSMAWYRQAPGKQRELVAAITGGGSPNYADSVKGRFTISSDVAKRTVYLQMNSLKPEDTAVYYCNAEGQAGWGTALMDYWGKGTLVTVSSRTVAAPSVFIFPPSDEQLKSGTASVVCLLNNFYPREAKVQWKVDNALQSGNSQESVTEQDSKDSTYSLSSTLTLSKADYEKHKVYACEVTHQGLSSPVTKSFNRGEC

SEQ ID NO: 230 - protein, 470 aa, Artificial Sequence
  Nanobody Chimera Sequence
MEWSWVFLFFLSVTTGVHSEVQLVESGGGLVQPGGSLRLSCAASETIFSIDSMAWYRQAPGKQRELVAAITGGGSPNYADSVKGRFTISSDVAKRTVYLQMNSLKPEDTAVYYCNAEGQAGWGTALMDYWGKGTLVTVSSASTKGPSVFPLAPSSKSTSGGTAALGCLVKDYFPEPVTVSWNSGALTSGVHTFPAVLQSSGLYSLSSVVTVPSSSLGTQTYICNVNHKPSNTKVDKKVEPKSCDKTHTCPPCPAPELLGGPSVFLFPPKPKDTLMISRTPEVTCVVVDVSHEDPEVKFNWYVDGVEVHNAKTKPREEQYNSTYRVVSVLTVLHQDWLNGKEYKCKVSNKALPAPIEKTISKAKGQPREPQVYTLPPSRDELTKNQVSLTCLVKGFYPSDIAVEWESNGQPENNYKTTPPVLDSDGSFFLYSKLTVDKSRWQQGNVFSCSVMHEALHNHYTQKSLSLSPGK

SEQ ID NO: 231 - protein, 241 aa, Homo sapiens
MAQHGAMGAFRALCGLALLCALSLGQRPTGGPGCGPGRLLLGTGTDARCCRVHTTRCCRDYPGEECCSEWDCMCVQPEFHCGDPCCTTCRHHPCPPGQGVQSQGKFSFGFQCIDCASGTFSGGHEGHCKPWTDCTQFGFLTVFPGNKTHNAVCVPGSPPAEPLGWLTVVLLAVAACVLLLTSAQLGLHIWQLRSQCMWPRETQLLLEVPPSTEDARSCQFPEEERGERSAEEKGRLGDLWV

SEQ ID NO: 232 - protein, 228 aa, Mus musculus
MGAWAMLYGVSMLCVLDLGQPSVVEEPGCGPGKVQNGSGNNTRCCSLYAPGKEDCPKERCICVTPEYHCGDPQCKICKHYPCQPGQRVESQGDIVFGFRCVACAMGTFSAGRDGHCRLWTNCSQFGFLTMFPGNKTHNAVCIPEPLPTEQYGHLTVIFLVMAACIFFLTTVQLGLHIWQLRRQHMCPRETQPFAEVQLSAEDACSFQFPEEERGEQTEEKCHLGGRWP

SEQ ID NO: 233 - protein, 235 aa, Macaca fascicularis
MCACGTLCCLALLCAASLGQRPTGGPGCGPGRLLLGTGKDARCCRVHPTRCCRDYQSEECCSEWDCVCVQPEFHCGNPCCTTCQHHPCPSGQGVQPQGKFSFGFRCVDCALGTFSRGHDGHCKPWTDCTQFGFLTVFPGNKTHNAVCVPGSPPAEPPGWLTIVLLAVAACVLLLTSAQLGLHIWQLGSQPTGPRETQLLLEVPPSTEDASSCQFPEEERGERLAEEKGRLGDLWV

SEQ ID NO: 234 - protein, 115 aa, Artificial Sequence [sequence omitted]

SEQ ID NO: 235 - protein, 115 aa, Artificial Sequence [sequence omitted]

SEQ ID NO: 236 - protein, 116 aa, Artificial Sequence
  Nanobody Sequence
EVQLVESGGGVVQPGNSLRLSCAASGFTFSSFGMSWVRQAPGKGLEWVSSISGSGSDTLYADSVKGRFTISRDNAKTTLYLQMNSLRPEDTATYYCTIGGSLSRSSQGTLVTVSSA

SEQ ID NO: 237 - protein, 116 aa, Artificial Sequence
  Nanobody Sequence
EVQLVESGGGVVQPGGSLRLSCAASGFTFRSFGMSWVRQAPGKGPEWVSSISGSGSDTLYADSVKGRFTISRDNSKNTLYLQMNSLRPEDTATYYCTIGGSLSRSSQGTLVTVSSA

SEQ ID NO: 238 - protein, 115 aa, Artificial Sequence [sequence omitted]

SEQ ID NO: 239 - protein, 116 aa, Artificial Sequence
  Nanobody Sequence
EVQLVESGGGLVQPGNSLRLSCAASGFTFSSFGMSWVRQAPGKGLEWVSSISGSGSDTLYADSVKGRFTISRDNAKTTLYLQMNSLRPEDTAVYYCTIGGSLSRSSQGTLVKVSSA

SEQ ID NO: 240 - protein, 115 aa, Artificial Sequence
  Nanobody Sequence
EVQLVESGGGVVQPGNSLRLSCAASGFTFSSFGMSWVRQAPGKGLEWVSSISGSGSDTLYADSVKGRFTISRDNAKTTLYLQMNSLRPEDTALYYCTIGGSLSRSSQGTLVTVSS

SEQ ID NO: 241 - protein, 116 aa, Artificial Sequence
  Nanobody Sequence
EVQLVESGGGVVQPGNSLRLSCAASGFTFSSFGMSWVRQAPGKGLEWVSSISGSGSDTLYADSVKGRFTISRDNAKTTLYLQMNSLRPEDTALYYCTIGGSLSRSSQGTLVTVSSA

SEQ ID NO: 242 - protein, 117 aa, Artificial Sequence
  Nanobody Sequence
EVQLVESGGGVVQPGNSLRLSCAASGFTFSSFGMSWVRQAPGKGLEWVSSISGSGSDTLYADSVKGRFTISRDNAKTTLYLQMNSLRPEDTALYYCTIGGSLSRSSQGTLVTVSSAA

SEQ ID NO: 243 - protein, 118 aa, Artificial Sequence
  Nanobody Sequence
EVQLVESGGGVVQPGNSLRLSCAASGFTFSSFGMSWVRQAPGKGLEWVSSISGSGSDTLYADSVKGRFTISRDNAKTTLYLQMNSLRPEDTALYYCTIGGSLSRSSQGTLVTVSSAAA

SEQ ID NO: 244 - protein, 116 aa, Artificial Sequence
  Nanobody Sequence
EVQLVESGGGVVQPGNSLRLSCAASGFTFSSFGMSWVRQAPGKGLEWVSSISGSGSDTLYADSVKGRFTISRDNAKTTLYLQMNSLRPEDTALYYCTIGGSLSRSSQGTLVTVSSG

SEQ ID NO: 245 - protein, 117 aa, Artificial Sequence
  Nanobody Sequence
EVQLVESGGGVVQPGNSLRLSCAASGFTFSSFGMSWVRQAPGKGLEWVSSISGSGSDTLYADSVKGRFTISRDNAKTTLYLQMNSLRPEDTALYYCTIGGSLSRSSQGTLVTVSSGG

SEQ ID NO: 246 - protein, 118 aa, Artificial Sequence
  Nanobody Sequence
EVQLVESGGGVVQPGNSLRLSCAASGFTFSSFGMSWVRQAPGKGLEWVSSISGSGSDTLYADSVKGRFTISRDNAKTTLYLQMNSLRPEDTALYYCTIGGSLSRSSQGTLVTVSSGGG

SEQ ID NO: 247 - protein, 3 aa, Artificial Sequence
  Linker
AAA

SEQ ID NO: 248 - protein, 5 aa, Artificial Sequence
  Linker
GGGGS

SEQ ID NO: 249 - protein, 7 aa, Artificial Sequence
  Linker
SGGSGGS

SEQ ID NO: 250 - protein, 9 aa, Artificial Sequence
  Linker
GGGGCGGGS

SEQ ID NO: 251 - protein, 9 aa, Artificial Sequence
  Linker
GGGGSGGGS

SEQ ID NO: 252 - protein, 10 aa, Artificial Sequence
  Linker
GGGGSGGGGS

SEQ ID NO: 253 - protein, 15 aa, Artificial Sequence
  Linker
GGGGSGGGGSGGGGS

SEQ ID NO: 254 - protein, 18 aa, Artificial Sequence
  Linker
GGGGSGGGGSGGGGGGGS

SEQ ID NO: 255 - protein, 20 aa, Artificial Sequence
  Linker
GGGGSGGGGSGGGGSGGGGS

SEQ ID NO: 256 - protein, 25 aa, Artificial Sequence
  Linker
GGGGSGGGGSGGGGSGGGGSGGGGS

SEQ ID NO: 257 - protein, 30 aa, Artificial Sequence
  Linker
GGGGSGGGGSGGGGSGGGGSGGGGSGGGGS

SEQ ID NO: 258 - protein, 35 aa, Artificial Sequence
  Linker
GGGGSGGGGSGGGGSGGGGSGGGGSGGGGSGGGGS

SEQ ID NO: 259 - protein, 40 aa, Artificial Sequence
  Linker
GGGGSGGGGSGGGGSGGGGSGGGGSGGGGSGGGGSGGGGS

SEQ ID NO: 260 - protein, 15 aa, Artificial Sequence
  Linker
EPKSCDKTHTCPPCP

SEQ ID NO: 261 - protein, 24 aa, Artificial Sequence
  Linker
GGGGSGGGSEPKSCDKTHTCPPCP

SEQ ID NO: 262 - protein, 12 aa, Artificial Sequence
  Linker
EPKTPKPQPAAA

SEQ ID NO: 263 - protein, 62 aa, Artificial Sequence
  Linker
ELKTPLGDTTHTCPRCPEPKSCDTPPPCPRCPEPKSCDTPPPCPRCPEPKSCDTPPPCPRCP

SEQ ID NO: 264 - protein, 115 aa, Artificial Sequence
  Nanobody
EVQLVESGGGVVQPGGSLRLSCAASGFTFRSFGMSWVRQAPGKGPEWVSSISGSGSDTLYADSVKGRFTISRDNSKNTLYLQMNSLRPEDTALYYCTIGGSLSRSSQGTLVTVSS

SEQ ID NO: 265 - protein, 116 aa, Artificial Sequence
  Nanobody
EVQLVESGGGVVQPGGSLRLSCAASGFTFRSFGMSWVRQAPGKGPEWVSSISGSGSDTLYADSVKGRFTISRDNSKNTLYLQMNSLRPEDTALYYCTIGGSLSRSSQGTLVTVSSA

SEQ ID NO: 266 - protein, 245 aa, Artificial Sequence
  Nanobody Chimera Sequence
MSVPTQVLGLLLLWLTDARCEVQLVESGGGLVQPGGSLRLSCAASETIFSIDSMAWYRQAPGKQRELVAAITGGGSPNYADSVKGRFTISSDVAKRTVYLQMNSLKPEDTAVYYCNAEGQAGWGTALMDYWGKGTLVTVSSQPKSTPQLTVFPPSTEELQGNKATLVCLISDFYPSDVEVAWKANGAPISQGVDTANPTKQGNKYIASSFLRLTAEQWRSRNSFTCQVTHEGNTVEKSLSPAECV

SEQ ID NO: 267 - protein, 473 aa, Artificial Sequence
  Nanobody Chimera Sequence
MEWSWVFLFFLSVTTGVHSEVQLVESGGGLVQPGGSLRLSCAASETIFSIDSMAWYRQAPGKQRELVAAITGGGSPNYADSVKGRFTISSDVAKRTVYLQMNSLKPEDTAVYYCNAEGQAGWGTALMDYWGKGTLVTVSSAQTTAPSVYPLAPGCGDTTSSTVTLGCLVKGYFPEPVTVTWNSGALSSDVHTFPAVLQSGLYTLTSSVTSSTWPSQTVTCNVAHPASSTKVDKKVERRNGGIGHKCPTCPTCHKCPVPELLGGPSVFIFPPKPKDILLISQNAKVTCVVVDVSEEEPDVQFSWFVNNVEVHTAQTQPREEQYNSTFRVVSALPIQHQDWMSGKEFKCKVNNKALPSPIEKTISKPKGLVRKPQVYVMGPPTEQLTEQTVSLTCLTSGFLPNDIGVEWTSNGHIEKNYKNTEPVMDSDGSFFMYSKLNVERSRWDSRAPFVCSVVHEGLHNHHVEKSISRPPGK

SEQ ID NO: 268 - protein, 115 aa, Artificial Sequence
  Nanobody Sequence
EVQLVESGGGVVQPGGSLRLSCTGSRSIFSTYAMAWHRQAPGKQRELVGFIYWGGTTTYADSVKGRFTISRDNSKNTLYLQMNSLRPEDTALYYCNIYGSYALPWGQGTLVTVSS

SEQ ID NO: 269 - protein, 119 aa, Artificial Sequence
  Nanobody Sequence
EVQLVESGGGVVQPGGSLRLSCAASGSIFSIDSMGWYRQAPGKQRELVAAITSSTNYADSVKGRFTISRDNSKNTVYLQMNSLRPEDTALYYCNLEGQAGWGTALINYWGQGTLVTVSS

SEQ ID NO: 270 - protein, 121 aa, Artificial Sequence
  Nanobody Sequence
EVQLVESGGGVVQPGGSLRLSCAASGSVFSINDMGWFRQAPGKQRELVADIISRGVTNYADSVKGRFTISGDPSKNTVYLQMNSLRPEDTALYYCNAHISTGWGRPHNNYWGQGTLVTVSS

SEQ ID NO: 271 - protein, 121 aa, Artificial Sequence
  Nanobody Sequence
EVQLVESGGGVVQPGGSLRLSCAASETIFSIDSMAWYRQAPGKQRELVAAITGGGSPNYADSVKGRFTISSDVSKRTVYLQMNSLRPEDTALYYCNAEGQAGWGTALMDYWGQGTLVTVSS

SEQ ID NO: 272 - protein, 121 aa, Artificial Sequence
  Nanobody Sequence
EVQLVESGGGVVQPGGSLRLSCAASETIFSIDSMAWYRQAPGKQRELVAAITGGGSPNYADSVKGRFTISSDVSKRTVYLQMNSLRPEDTALYYCNAEGQAGWGTALLDYWGQGTLVTVSS

SEQ ID NO: 273 - protein, 121 aa, Artificial Sequence
  Nanobody Sequence
EVQLVESGGGVVQPGGSLRLSCAASETIFSIDSMAWYRQAPGKQRELVAAITGGGSPNYADSVKGRFTISSDVSKRTVYLQMNSLRPEDTALYYCNAEGQAGWGTALKDYWGQGTLVTVSS

SEQ ID NO: 274 - protein, 121 aa, Artificial Sequence
  Nanobody Sequence
EVQLVESGGGVVQPGGSLRLSCAASETIFSIDSMAWYRQAPGKQRELVAAITGGGSPNYADSVKGRFTISSDVSKRTVYLQMNSLRPEDTALYYCNAEGQAGWGTALRDYWGQGTLVTVSS

SEQ ID NO: 275 - protein, 121 aa, Artificial Sequence
  Nanobody Sequence
EVQLVESGGGVVQPGGSLRLSCAASETIFSIDSMAWYRQAPGKQRELVAAITGGGSPNYADSVKGRFTISSDVSKRTVYLQMNSLRPEDTALYYCNAEGQAGWGTALQDYWGQGTLVTVSS

SEQ ID NO: 276 - protein, 25 aa, Artificial Sequence
  FR1
EVQLVESGGGVVQPGGSLRLSCTGS

SEQ ID NO: 277 - protein, 39 aa, Artificial Sequence
  FR3
YADSVKGRFTISRDNSKNTLYLQMNSLRPEDTALYYCNI

SEQ ID NO: 278 - protein, 25 aa, Artificial Sequence
  FR1
EVQLVESGGGVVQPGGSLRLSCAAS

SEQ ID NO: 279 - protein, 39 aa, Artificial Sequence
  FR3
YADSVKGRFTISRDNSKNTVYLQMNSLRPEDTALYYCNL

SEQ ID NO: 280 - protein, 39 aa, Artificial Sequence
  FR3
YADSVKGRFTISGDPSKNTVYLQMNSLRPEDTALYYCNA

SEQ ID NO: 281 - protein, 39 aa, Artificial Sequence
  FR3
YADSVKGRFTISSDVSKRTVYLQMNSLRPEDTALYYCNA

SEQ ID NO: 282 - protein, 13 aa, Artificial Sequence
  CDR3
EGQAGWGTALKDY

SEQ ID NO: 283 - protein, 13 aa, Artificial Sequence
  CDR3
EGQAGWGTALRDY

SEQ ID NO: 284 - protein, 13 aa, Artificial Sequence
  CDR3
EGQAGWGTALQDY

SEQ ID NO: 285 - protein, 532 aa, Artificial Sequence
  Nanobody Sequence
DVQLVESGGGVVQPGGSLRLSCAASETIFSIDSMAWYRQAPGKQRELVAAITGGGSPNYADSVKGRFTISSDVSKRTVYLQMNSLRPEDTALYYCNAEGQAGWGTALLDYWGQGTLVTVSSGGGGSGGGSEVQLVESGGGVVQPGGSLRLSCAASETIFSIDSMAWYRQAPGKQRELVAAITGGGSPNYADSVKGRFTISSDVSKRTVYLQMNSLRPEDTALYYCNAEGQAGWGTALLDYWGQGTLVTVSSGGGGSGGGSEVQLVESGGGVVQPGGSLRLSCAASETIFSIDSMAWYRQAPGKQRELVAAITGGGSPNYADSVKGRFTISSDVSKRTVYLQMNSLRPEDTALYYCNAEGQAGWGTALLDYWGQGTLVTVSSGGGGSGGGGSGGGGSGGGGSGGGGSGGGGSGGGGSEVQLVESGGGVVQPGGSLRLSCAASGFTFRSFGMSWVRQAPGKGPEWVSSISGSGSDTLYADSVKGRFTISRDNSKNTLYLQMNSLRPEDTALYYCTIGGSLSRSSQGTLVTVSSA

SEQ ID NO: 286 - protein, 526 aa, Artificial Sequence
  Nanobody Sequence
DVQLVESGGGVVQPGGSLRLSCAASGSIFSIDSMGWYRQAPGKQRELVAAITSSTNYADSVKGRFTISRDNSKNTVYLQMNSLRPEDTALYYCNLEGQAGWGTALINYWGQGTLVTVSSGGGGSGGGSEVQLVESGGGVVQPGGSLRLSCAASGSIFSIDSMGWYRQAPGKQRELVAAITSSTNYADSVKGRFTISRDNSKNTVYLQMNSLRPEDTALYYCNLEGQAGWGTALINYWGQGTLVTVSSGGGGSGGGSEVQLVESGGGVVQPGGSLRLSCAASGSIFSIDSMGWYRQAPGKQRELVAAITSSTNYADSVKGRFTISRDNSKNTVYLQMNSLRPEDTALYYCNLEGQAGWGTALINYWGQGTLVTVSSGGGGSGGGGSGGGGSGGGGSGGGGSGGGGSGGGGSEVQLVESGGGVVQPGGSLRLSCAASGFTFRSFGMSWVRQAPGKGPEWVSSISGSGSDTLYADSVKGRFTISRDNSKNTLYLQMNSLRPEDTALYYCTIGGSLSRSSQGTLVTVSSA

SEQ ID NO: 287 - protein, 662 aa, Artificial Sequence
  Nanobody Sequence
DVQLVESGGGVVQPGGSLRLSCAASETIFSIDSMAWYRQAPGKQRELVAAITGGGSPNYADSVKGRFTISSDVSKRTVYLQMNSLRPEDTALYYCNAEGQAGWGTALLDYWGQGTLVTVSSGGGGSGGGSEVQLVESGGGVVQPGGSLRLSCAASETIFSIDSMAWYRQAPGKQRELVAAITGGGSPNYADSVKGRFTISSDVSKRTVYLQMNSLRPEDTALYYCNAEGQAGWGTALLDYWGQGTLVTVSSGGGGSGGGSEVQLVESGGGVVQPGGSLRLSCAASETIFSIDSMAWYRQAPGKQRELVAAITGGGSPNYADSVKGRFTISSDVSKRTVYLQMNSLRPEDTALYYCNAEGQAGWGTALLDYWGQGTLVTVSSGGGGSGGGSEVQLVESGGGVVQPGGSLRLSCAASETIFSIDSMAWYRQAPGKQRELVAAITGGGSPNYADSVKGRFTISSDVSKRTVYLQMNSLRPEDTALYYCNAEGQAGWGTALLDYWGQGTLVTVSSGGGGSGGGGSGGGGSGGGGSGGGGSGGGGSGGGGSEVQLVESGGGVVQPGGSLRLSCAASGFTFRSFGMSWVRQAPGKGPEWVSSISGSGSDTLYADSVKGRFTISRDNSKNTLYLQMNSLRPEDTALYYCTIGGSLSRSSQGTLVTVSSA

SEQ ID NO: 288 - protein, 792 aa, Artificial Sequence
  Nanobody Sequence
DVQLVESGGGVVQPGGSLRLSCAASETIFSIDSMAWYRQAPGKQRELVAAITGGGSPNYADSVKGRFTISSDVSKRTVYLQMNSLRPEDTALYYCNAEGQAGWGTALLDYWGQGTLVTVSSGGGGSGGGSEVQLVESGGGVVQPGGSLRLSCAASETIFSIDSMAWYRQAPGKQRELVAAITGGGSPNYADSVKGRFTISSDVSKRTVYLQMNSLRPEDTALYYCNAEGQAGWGTALLDYWGQGTLVTVSSGGGGSGGGSEVQLVESGGGVVQPGGSLRLSCAASETIFSIDSMAWYRQAPGKQRELVAAITGGGSPNYADSVKGRFTISSDVSKRTVYLQMNSLRPEDTALYYCNAEGQAGWGTALLDYWGQGTLVTVSSGGGGSGGGSEVQLVESGGGVVQPGGSLRLSCAASETIFSIDSMAWYRQAPGKQRELVAAITGGGSPNYADSVKGRFTISSDVSKRTVYLQMNSLRPEDTALYYCNAEGQAGWGTALLDYWGQGTLVTVSSGGGGSGGGSEVQLVESGGGVVQPGGSLRLSCAASETIFSIDSMAWYRQAPGKQRELVAAITGGGSPNYADSVKGRFTISSDVSKRTVYLQMNSLRPEDTALYYCNAEGQAGWGTALLDYWGQGTLVTVSSGGGGSGGGGSGGGGSGGGGSGGGGSGGGGSGGGGSEVQLVESGGGVVQPGGSLRLSCAASGFTFRSFGMSWVRQAPGKGPEWVSSISGSGSDTLYADSVKGRFTISRDNSKNTLYLQMNSLRPEDTALYYCTIGGSLSRSSQGTLVTVSSA

SEQ ID NO: 289 - protein, 654 aa, Artificial Sequence
  Nanobody Sequence
DVQLVESGGGVVQPGGSLRLSCAASGSIFSIDSMGWYRQAPGKQRELVAAITSSTNYADSVKGRFTISRDNSKNTVYLQMNSLRPEDTALYYCNLEGQAGWGTALINYWGQGTLVTVSSGGGGSGGGSEVQLVESGGGVVQPGGSLRLSCAASGSIFSIDSMGWYRQAPGKQRELVAAITSSTNYADSVKGRFTISRDNSKNTVYLQMNSLRPEDTALYYCNLEGQAGWGTALINYWGQGTLVTVSSGGGGSGGGSEVQLVESGGGVVQPGGSLRLSCAASGSIFSIDSMGWYRQAPGKQRELVAAITSSTNYADSVKGRFTISRDNSKNTVYLQMNSLRPEDTALYYCNLEGQAGWGTALINYWGQGTLVTVSSGGGGSGGGSEVQLVESGGGVVQPGGSLRLSCAASGSIFSIDSMGWYRQAPGKQRELVAAITSSTNYADSVKGRFTISRDNSKNTVYLQMNSLRPEDTALYYCNLEGQAGWGTALINYWGQGTLVTVSSGGGGSGGGGSGGGGSGGGGSGGGGSGGGGSGGGGSEVQLVESGGGVVQPGGSLRLSCAASGFTFRSFGMSWVRQAPGKGPEWVSSISGSGSDTLYADSVKGRFTISRDNSKNTLYLQMNSLRPEDTALYYCTIGGSLSRSSQGTLVTVSSA

SEQ ID NO: 290 - protein, 782 aa, Artificial Sequence
  Nanobody Sequence
DVQLVESGGGVVQPGGSLRLSCAASGSIFSIDSMGWYRQAPGKQRELVAAITSSTNYADSVKGRFTISRDNSKNTVYLQMNSLRPEDTALYYCNLEGQAGWGTALINYWGQGTLVTVSSGGGGSGGGSEVQLVESGGGVVQPGGSLRLSCAASGSIFSIDSMGWYRQAPGKQRELVAAITSSTNYADSVKGRFTISRDNSKNTVYLQMNSLRPEDTALYYCNLEGQAGWGTALINYWGQGTLVTVSSGGGGSGGGSEVQLVESGGGVVQPGGSLRLSCAASGSIFSIDSMGWYRQAPGKQRELVAAITSSTNYADSVKGRFTISRDNSKNTVYLQMNSLRPEDTALYYCNLEGQAGWGTALINYWGQGTLVTVSSGGGGSGGGSEVQLVESGGGVVQPGGSLRLSCAASGSIFSIDSMGWYRQAPGKQRELVAAITSSTNYADSVKGRFTISRDNSKNTVYLQMNSLRPEDTALYYCNLEGQAGWGTALINYWGQGTLVTVSSGGGGSGGGSEVQLVESGGGVVQPGGSLRLSCAASGSIFSIDSMGWYRQAPGKQRELVAAITSSTNYADSVKGRFTISRDNSKNTVYLQMNSLRPEDTALYYCNLEGQAGWGTALINYWGQGTLVTVSSGGGGSGGGGSGGGGSGGGGSGGGGSGGGGSGGGGSEVQLVESGGGVVQPGGSLRLSCAASGFTFRSFGMSWVRQAPGKGPEWVSSISGSGSDTLYADSVKGRFTISRDNSKNTLYLQMNSLRPEDTALYYCTIGGSLSRSSQGTLVTVSSA

SEQ ID NO: 291 - protein, 248 aa, Artificial Sequence
  Nanobody Chimera Sequence
MSVPTQVLGLLLLWLTDARCEVQLVESGGGVVQPGGSLRLSCAASETIFSIDSMAWYRQAPGKQRELVAAITGGGSPNYADSVKGRFTISSDVSKRTVYLQMNSLRPEDTALYYCNAEGQAGWGTALLDYWGQGTLVTVSSRTVAAPSVFIFPPSDEQLKSGTASVVCLLNNFYPREAKVQWKVDNALQSGNSQESVTEQDSKDSTYSLSSTLTLSKADYEKHKVYACEVTHQGLSSPVTKSFNRGEC

SEQ ID NO: 292 - protein, 470 aa, Artificial Sequence
  Nanobody Chimera Sequence
MEWSWVFLFFLSVTTGVHSEVQLVESGGGVVQPGGSLRLSCAASETIFSIDSMAWYRQAPGKQRELVAAITGGGSPNYADSVKGRFTISSDVSKRTVYLQMNSLRPEDTALYYCNAEGQAGWGTALLDYWGQGTLVTVSSASTKGPSVFPLAPSSKSTSGGTAALGCLVKDYFPEPVTVSWNSGALTSGVHTFPAVLQSSGLYSLSSVVTVPSSSLGTQTYICNVNHKPSNTKVDKKVEPKSCDKTHTCPPCPAPELLGGPSVFLFPPKPKDTLMISRTPEVTCVVVDVSHEDPEVKFNWYVDGVEVHNAKTKPREEQYNSTYRVVSVLTVLHQDWLNGKEYKCKVSNKALPAPIEKTISKAKGQPREPQVYTLPPSRDELTKNQVSLTCLVKGFYPSDIAVEWESNGQPENNYKTTPPVLDSDGSFFLYSKLTVDKSRWQQGNVFSCSVMHEALHNHYTQKSLSLSPGK